European Patent Specification EP 3 024 929 B1, published October 16, 2024. Title: DOWNY MILDEW RESISTANCE PROVIDING GENES IN SUNFLOWER. Applicant: SciENZA Biotechnologies 5 B.V. Application EP14741337.1. The sequence listing filed with the application follows.

SEQUENCE LISTING (4 sequences)

SEQ ID NO: 1 - DNA, 1014 bp, Helianthus annuus
  source 1..1014: /mol_type="unassigned DNA" /note="HaTZ1" /organism="Helianthus annuus"
atggcgggaaaagtcatctccagtggcatccaatacactactttacccgacagttacgtccgtccggtcaacgacaggcctaacctatcccaagtctccgaatgcaacgatgttccggttatcgacatcggtggagctgaccgggagctcataagccggcaaatcggcgatgcgtgccgtcactacggctttttccaggtgataaaccacggtgtggcggatgaattggtgaagaagatggagcaggtagggagagatttcttccagttgccggttgaggagaagatgaagctctactcggaggatccgacgaagacgatgaggctttcgacgagcttcaacgtcaagaaagaacaagtgcataactggagggattatctccggcttcactgctatcctttggatcagtactctcctgaatggccttccaatccttgttatttcaaagaatatgttggaaattactgtatagcggtacgcgaattagggatgaggatacttgaattcatatcggaaagtttaggtttagaaaaagagcgactaaatatgatattaggcgagcaaggacaacatatggccatcaaccattatccagtgtgccctgaacctgagttaacttatgggttgcctggtcacactgatcctaatgcactcaccatactccttcaagacacgcttgtctctggattacaagttcaaaaagatggcaaatgggtagcggttaaaccacaccctaacgcgtttgtcatcaacattggcgaccaactagaggcgttgagtaatggtgaatacaagagtgtgtggcatcgagccgtggtcaactcagaccaaccaagaatgtcaatagcttcgtttttgtgtccctgtaatgactcagtcctcagcgctcctaacgaactaataaaagatggatcgacgcgtgttttcaaagactttacttacacagaatactacaagaagttttggagtcgaaatctagaccaagaacattgtttagagttcttcaagaactag

SEQ ID NO: 2 - protein, 337 aa, Helianthus annuus
  HaTZ1
MAGKVISSGIQYTTLPDSYVRPVNDRPNLSQVSECNDVPVIDIGGADRELISRQIGDACRHYGFFQVINHGVADELVKKMEQVGRDFFQLPVEEKMKLYSEDPTKTMRLSTSFNVKKEQVHNWRDYLRLHCYPLDQYSPEWPSNPCYFKEYVGNYCIAVRELGMRILEFISESLGLEKERLNMILGEQGQHMAINHYPVCPEPELTYGLPGHTDPNALTILLQDTLVSGLQVQKDGKWVAVKPHPNAFVINIGDQLEALSNGEYKSVWHRAVVNSDQPRMSIASFLCPCNDSVLSAPNELIKDGSTRVFKDFTYTEYYKKFWSRNLDQEHCLEFFKN

SEQ ID NO: 3 - DNA, 1035 bp, Helianthus annuus
  source 1..1035: /mol_type="unassigned DNA" /note="HaTZ2" /organism="Helianthus annuus"
atggctaccacctcaaaaagattactagttagcgacctcgtatccaccgataaaatcgaccaagtcccttcaaactacatccgacccatcacccaacgtcccaatttccaaaatgttgttcgcgactccatccctctcattgacctcaaagatctcaacggccccaatcacgctaacgtgatcaaacaaatcggtcaagcttgcgctgatcacggcttcttccaggttaaaaaccatggcgtacccgaatccatcatagccaacatgatgcaaaccgctcgagacttcttcaacctacccgaacaagaacgactcaaaaactattcagatgaccccacaaagaccactagactctccaccagcttcaacatacgaaccgaaaaggtcgcaaactggagagattacttacgactccattgctacccgatcgataacttcatcgacgaatggccaaccaatccggcctcgtttcgggcccatgtagcggagtattgccagagtacaagaaacttagcactccaacttattgcagccatttcagaaagcttaggacttcataaagactacatgaacacacagttagggaagcatgctcagcatatggtcttgaactactacccaccatgcccacaacccgatttaacatacgggttacccggacacactgatcctaatttcatcaccatccttcttcaagatgaggttcctggtcttcaggtcttgaaagatggtaaatgggtagcggttgatccggttccaaacactttcatcatcaacattggtgatcaagttcaggtgatgagtaatgataagtacaagagtattttgcatcgagctgtggtgaattgtgataaagaacggatatctataccgactttctactgtccgtcgcctgaggcggttatcgggcctgctcccgaggttgtaactgatgatgagcctgctgtgtatcgacagtttacttatggggagtactatgagaagttttgggacaatgggcttgagaagtgtttggatatgttcaagactagttga

SEQ ID NO: 4 - protein, 344 aa, Helianthus annuus
  HaTZ2
MATTSKRLLVSDLVSTDKIDQVPSNYIRPITQRPNFQNVVRDSIPLIDLKDLNGPNHANVIKQIGQACADHGFFQVKNHGVPESIIANMMQTARDFFNLPEQERLKNYSDDPTKTTRLSTSFNIRTEKVANWRDYLRLHCYPIDNFIDEWPTNPASFRAHVAEYCQSTRNLALQLIAAISESLGLHKDYMNTQLGKHAQHMVLNYYPPCPQPDLTYGLPGHTDPNFITILLQDEVPGLQVLKDGKWVAVDPVPNTFIINIGDQVQVMSNDKYKSILHRAVVNCDKERISIPTFYCPSPEAVIGPAPEVVTDDEPAVYRQFTYGEYYEKFWDNGLEKCLDMFKTS